European Patent Specification EP 3 347 380 B1, published September 25, 2024. Title: Enhanced Delivery of Drugs to the Brain. Applicant: Nascent Biotech Inc. The sequence listing filed with the application follows.

SEQUENCE LISTING (55 sequences)

SEQ ID NO: 1 - protein, 450 aa, Artificial Sequence
  Synthetic Construct
EVQLLESGGDLVQPGGSLRLSCAASGFTFSNYAMSWVRQAPGKGLEWVSAITPSGGSTNYADSVKGRFTISRDNSQNTLYLQMNSLRVEDTAVYICGRVPYRSTWYPLYWGQGTLVTVSSASTKGPSVFPLAPSSKSTSGGTAALGCLVKDYFPEPVTVSWNSGALTSGVHTFPAVLQSSGLYSLSSVVTVPSSSLGTQTYICNVNHKPSNTKVDKKVEPKSCDKTHTCPPCPAPELLGGPSVFLFPPKPKDTLMISRTPEVTCVVVDVSHEDPEVKFNWYVDGVEVHNAKTKPREEQYNSTYRVVSVLTVLHQDWLNGKEYKCKVSNKALPAPIEKTISKAKGQPREPQVYTLPPSRDELTKNQVSLTCLVKGFYPSDIAVEWESNGQPENNYKTTPPVLDSDGSFFLYSKLTVDKSRWQQGNVFSCSVMHEALHNHYTQKSLSLSPGK

SEQ ID NO: 2 - protein, 214 aa, Artificial Sequence
  Synthetic Construct
DIQMTQSPSSLSASVGDRVTITCRASQDISNYLAWFQQKPGKAPKSLIYAASSLHSKVPTQFSGSGSGTDFTLTISSLQPEDFATYYCLQYSTYPITFGGGTKVEIKRTVAAPSVFIFPPSDEQLKSGTASVVCLLNNFYPREAKVQWKVDNALQSGNSQESVTEQDSKDSTYSLSSTLTLSKADYEKHKVYACEVTHQGLSSPVTKSFNRGEC

SEQ ID NO: 3 - protein, 226 aa, ARTIFICIAL SEQUENCE
  SYNTHETIC CONSTRUCT
QVQLKQSGPGLVQPSQSLSITCTVSGFSLTNYGVHWVRQSPGKGLEWLGVIWSGGNTDYNTPFTSRLSINKDNSKSQVFFKMNSLQSNDTAIYYCARALTYYDYEFAYWGQGTLVTVSADILLTQSPVILSVSPGERVSFSCRASQSIGTNIHWYQQRTNGSPRLLIKYASESISGIPSRFSGSGSGTDFTLSINSVESEDIADYYCQQNNNWPTTFGAGTKLELK

SEQ ID NO: 4 - protein, 226 aa, ARTIFICIAL SEQUENCE
  SYNTHETIC CONSTRUCT
QVQLQQPGAELVKPGASVKMSCKASGYTFTSYNMHWVKQTPGRGLEWIGAIYPGNGDTSYNQKFKGKATLTADKSSSTAYMQLSSLTSEDSAVYYCARSTYYGGDWYFNVWGAGTTVTVSAQIVLSQSPAILSASPGEKVTMTCRASSSVSYIHWFQQKPGSSPKPWIYATSNLASGVPVRFSGSGSGTSYSLTISVEAEDAATYYCQQWTSNPPTFGGGTKLEIK

SEQ ID NO: 5 - protein, 228 aa, ARTIFICIAL SEQUENCE
  SYNTHETIC CONSTRUCT
QVQLQESGPGLVRPSQTLSLTCTVSGFTFTDFYMNWVRQPPGRGLEWIGFIRDKAKGYTTEYNPSVKGRVTMLVDTSKNQFSLRLSSVTAADTAVYYCAREGHTAAPFDYWGQGSLVTVSSDIQMTQSPSSLSASVGDRVTITCKASQNIDKYLNWYQQKPGKAPKLLIYNTNNLQTGVPSRFSGSGSGTDFTFTISSLQPEDIATYYCLQHISRPRTFGQGTKVEIK

SEQ ID NO: 6 - protein, 230 aa, ARTIFICIAL SEQUENCE
  SYNTHETIC CONSTRUCT
EVQLVESGGGLVQPGGSLRLSCAASGYTFTNYGMNWVRQAPGKGLEWVGWINTYTGEPTYAADFKRRFTFSLDTSKSTAYLQMNSLRAEDTAVYYCAKYPHYYGSSHWYFDVWGQGTLVTVSSDIQMTQSPSSLSASVGDRVTITCSASQDISNYLNWYQQKPGKAPKVLIYFTSSLHSGVPSRFSGSGSGTDFTLTISSLQPEDFATYYCQQYSTVPWTFGQGTKVEIK

SEQ ID NO: 7 - protein, 225 aa, ARTIFICIAL SEQUENCE
  SYNTHETIC CONSTRUCT
EVQLVESGGGLVQPGGSLRLSCAASGFNIKDTYIHWVRQAPGKGLEWVARIYPTNGYTRYADSVKGRFTISADTSKNTAYLQMNSLRAEDTAVYYCSRWGGDGFYAMDYWGQGTLVTVSSDIQMTQSPSSLSASVGDRVTITCRASQDVNTAVAWYQQKPGKAPKLLIYSASFLYGVPSRFGSRSGTDFTLTISSLQPEDFATYYCQQHYTTPPTFGQGTKVEIK

SEQ ID NO: 8 - protein, 226 aa, ARTIFICIAL SEQUENCE
  SYNTHETIC CONSTRUCT
EVQLVESGGGLVQPGGSLRLSCAASGFTFTDYTMDWVRQAPGKGLEWVADVNPNSGGSIYNQRFKGRFTLSVDRSKNTLYLQMNSLRAEDTAVYYCARNLGPSFYFDYWGQGTLVTVSSDIQMTQSPSSLSASVGDRVTITCKASQDVSIGVAWYQQKPGKAPKLLIYSASYRYTGVPSRFSGSGSGTDFTLTISSLQPEDFATYYCQQYYIYPYTFGQGTKVEIK

SEQ ID NO: 9 - protein, 184 aa, ARTIFICIAL SEQUENCE
  SYNTHETIC CONSTRUCT
VSGGSVSSGDYYWRWIRQSPGKGLEWIGHIYYSGNTNYNPSKLSRLTISIDTSKTQFSLKLSSVTAADTAIYYCVRDRVYGAFDIWGQGTMVTVSSTITDQASQDISNYLNWYQQKPGKAPKLLIYDASNLETGVPSRFSGSGSGTDFTFTISSLQPEDIATYFCQHFDHLPLAFGGGTKVEIK

SEQ ID NO: 10 - protein, 229 aa, ARTIFICIAL SEQUENCE
  SYNTHETIC CONSTRUCT
EVQLVESGGGLVQPGGSLRLSCAASGYTFTNYGMNWVRQAPGKGLEWVGWINTYTGEPTYAADFKRRFTSLDTSKSTAYLQMNSLRAEDTAVYYCAKYPHYYGSSHWYFDVWGQGTLVTVSSDIQMTQSPSSLSASVGDRVTITCSASQDISNYLNWYQQKPGKAPKVLIYFTSSLHSGVPSRFSGSGSGTDFTLTISSLQPEDFATYYCQQYSTVPWTFGQGTKVEIK

SEQ ID NO: 11 - protein, 229 aa, ARTIFICIAL SEQUENCE
  SYNTHETIC CONSTRUCT
EVQLVESGGGLVQPGGSLRLSCAASGYDFTHYGMNWVRQAPGKGLEWVGWINTYTGEPTYAADFKRRFTSLDTSKSTAYLQMNSLRAEDTAVYYCAKYPYYYGTSHWYFDVWGQGTLVTVSSDIQLTQSPSSLSASVGDRVTITCSASQDISNYLNWYQQKPGKAPKVLIYFTSSLHSGVPSRFSGSGSGTDFTLTISSLQPEDFATYYCQQYSTVPWTFGQGTKVEIK

SEQ ID NO: 12 - DNA, 20 bp, ARTIFICIAL SEQUENCE
  SYNTHETIC CONSTRUCT
tcaccttcagcaactatgcc

SEQ ID NO: 13 - DNA, 24 bp, ARTIFICIAL SEQUENCE
  SYNTHETIC CONSTRUCT
aagggtaccaagtgcttctatatg

SEQ ID NO: 14 - DNA, 20 bp, ARTIFICIAL SEQUENCE
  SYNTHETIC CONSTRUCT
gagtgggtctcagcgattac

SEQ ID NO: 15 - DNA, 18 bp, ARTIFICIAL SEQUENCE
  SYNTHETIC CONSTRUCT
agaggtgctcttggagga

SEQ ID NO: 16 - DNA, 18 bp, ARTIFICIAL SEQUENCE
  SYNTHETIC CONSTRUCT
ctatgccatgagctgggt

SEQ ID NO: 17 - DNA, 24 bp, ARTIFICIAL SEQUENCE
  SYNTHETIC CONSTRUCT
tctatatggactctcccacagata

SEQ ID NO: 18 - DNA, 20 bp, ARTIFICIAL SEQUENCE
  SYNTHETIC CONSTRUCT
gcctggtcaaaggcttctat

SEQ ID NO: 19 - DNA, 20 bp, ARTIFICIAL SEQUENCE
  SYNTHETIC CONSTRUCT
tcttctgcgtgtagtggttg

SEQ ID NO: 20 - DNA, 20 bp, ARTIFICIAL SEQUENCE
  SYNTHETIC CONSTRUCT
gctgaatggcaaggagtaca

SEQ ID NO: 21 - DNA, 22 bp, ARTIFICIAL SEQUENCE
  SYNTHETIC CONSTRUCT
gagcttgctgtagaggaagaag

SEQ ID NO: 22 - DNA, 22 bp, ARTIFICIAL SEQUENCE
  SYNTHETIC CONSTRUCT
caaggtggacaagaaagttgag

SEQ ID NO: 23 - DNA, 20 bp, ARTIFICIAL SEQUENCE
  SYNTHETIC CONSTRUCT
catcacggagcatgagaaga

SEQ ID NO: 24 - DNA, 18 bp, ARTIFICIAL SEQUENCE
  SYNTHETIC CONSTRUCT
atcacaagcccagcaaca

SEQ ID NO: 25 - DNA, 21 bp, ARTIFICIAL SEQUENCE
  SYNTHETIC CONSTRUCT
gaccttgcacttgtactcctt

SEQ ID NO: 26 - DNA, 20 bp, ARTIFICIAL SEQUENCE
  SYNTHETIC CONSTRUCT
gtgcaaggtctccaacaaag

SEQ ID NO: 27 - DNA, 22 bp, ARTIFICIAL SEQUENCE
  SYNTHETIC CONSTRUCT
gcgtggtcttgtagttgttctc

SEQ ID NO: 28 - DNA, 22 bp, ARTIFICIAL SEQUENCE
  SYNTHETIC CONSTRUCT
gcatctgtaggagacagagtca

SEQ ID NO: 29 - DNA, 22 bp, ARTIFICIAL SEQUENCE
  SYNTHETIC CONSTRUCT
gccgaaggtgatagggtaagta

SEQ ID NO: 30 - DNA, 20 bp, ARTIFICIAL SEQUENCE
  SYNTHETIC CONSTRUCT
agtctccatcctcactgtct

SEQ ID NO: 31 - DNA, 22 bp, ARTIFICIAL SEQUENCE
  SYNTHETIC CONSTRUCT
gagtgaaatctgtcccagatcc

SEQ ID NO: 32 - DNA, 22 bp, ARTIFICIAL SEQUENCE
  SYNTHETIC CONSTRUCT
gagacagagtcaccatcacttg

SEQ ID NO: 33 - DNA, 24 bp, ARTIFICIAL SEQUENCE
  SYNTHETIC CONSTRUCT
agggtaagtactatactgtaggca

SEQ ID NO: 34 - DNA, 21 bp, ARTIFICIAL SEQUENCE
  SYNTHETIC CONSTRUCT
ctgcaccatctgtcttcatct

SEQ ID NO: 35 - DNA, 21 bp, ARTIFICIAL SEQUENCE
  SYNTHETIC CONSTRUCT
aggcgtagactttgtgtttct

SEQ ID NO: 36 - DNA, 19 bp, ARTIFICIAL SEQUENCE
  SYNTHETIC CONSTRUCT
cttcatcttcccgccatct

SEQ ID NO: 37 - DNA, 22 bp, ARTIFICIAL SEQUENCE
  SYNTHETIC CONSTRUCT
gtgtttctcgtagtctgctttg

SEQ ID NO: 38 - DNA, 20 bp, ARTIFICIAL SEQUENCE
  SYNTHETIC CONSTRUCT
atctggaactgcctctgttg

SEQ ID NO: 39 - DNA, 19 bp, ARTIFICIAL SEQUENCE
  SYNTHETIC CONSTRUCT
cttcgcaggcgtagacttt

SEQ ID NO: 40 - DNA, 21 bp, ARTIFICIAL SEQUENCE
  SYNTHETIC CONSTRUCT
gttgtgtgcctgctgaataac

SEQ ID NO: 41 - DNA, 21 bp, ARTIFICIAL SEQUENCE
  SYNTHETIC CONSTRUCT
ccctgttgaagctctttgtga

SEQ ID NO: 42 - DNA, 21 bp, ARTIFICIAL SEQUENCE
  SYNTHETIC CONSTRUCT
aggtggagatcaaacgaactg

SEQ ID NO: 43 - DNA, 19 bp, ARTIFICIAL SEQUENCE
  SYNTHETIC CONSTRUCT
gctgtaggtgctgtccttg

SEQ ID NO: 44 - DNA, 21 bp, ARTIFICIAL SEQUENCE
  SYNTHETIC CONSTRUCT
gttatgcgcctgcgtctgtac

SEQ ID NO: 45 - DNA, 20 bp, ARTIFICIAL SEQUENCE
  SYNTHETIC CONSTRUCT
ccgggtgttcagaactcgtc

SEQ ID NO: 46 - DNA, 19 bp, ARTIFICIAL SEQUENCE
  SYNTHETIC CONSTRUCT
acggtgtcgtggaactcag

SEQ ID NO: 47 - DNA, 24 bp, ARTIFICIAL SEQUENCE
  SYNTHETIC CONSTRUCT
cacgctgctgagggagtagagtcc

SEQ ID NO: 48 - DNA, 22 bp, ARTIFICIAL SEQUENCE
  SYNTHETIC CONSTRUCT
caaagtacagtggaaggtggat

SEQ ID NO: 49 - DNA, 24 bp, ARTIFICIAL SEQUENCE
  SYNTHETIC CONSTRUCT
gtgctgtccttgctgtcctgctct

SEQ ID NO: 50 - DNA, 21 bp, ARTIFICIAL SEQUENCE
  SYNTHETIC CONSTRUCT
aaagatgggcggtcgttattc

SEQ ID NO: 51 - DNA, 24 bp, ARTIFICIAL SEQUENCE
  SYNTHETIC CONSTRUCT
cctgccggttgcgaaatgggataa

SEQ ID NO: 52 - DNA, 35 bp, ARTIFICIAL SEQUENCE
  SYNTHETIC CONSTRUCT
ttttaagcttgccgccaccatgatgtcctttgtct

SEQ ID NO: 53 - DNA, 71 bp, ARTIFICIAL SEQUENCE
  SYNTHETIC CONSTRUCT
gccagggggaagaccgatgggcccttggtggaggcagaggacacggtcacgagggtgccctggccccaata

SEQ ID NO: 54 - DNA, 71 bp, ARTIFICIAL SEQUENCE
  SYNTHETIC CONSTRUCT
tattggggccagggcaccctcgtgaccgtgtcctctgcctccaccaagggcccatcggtcttccccctggc

SEQ ID NO: 55 - DNA, 59 bp, ARTIFICIAL SEQUENCE
  SYNTHETIC CONSTRUCT
tttctcgagatctcatcatttcccgggagacagggagaggctcttctgcgtgtagtggt